European Patent Specification EP 3 866 850 B1, published July 24, 2024. Title: COMBINATION THERAPY FOR MELANOMA. Applicant: BRISTOL-MYERS SQUIBB COMPANY. The sequence listing filed with the application follows.

SEQUENCE LISTING (30 sequences)

SEQ ID NO: 1 - protein, 447 aa, Artificial Sequence
  Heavy Chain Amino Acid Sequence; Anti-LAG-3 mAb (BMS-986016)
QVQLQQWGAGLLKPSETLSLTCAVYGGSFSDYYWNWIRQPPGKGLEWIGEINHRGSTNSNPSLKSRVTLSLDTSKNQFSLKLRSVTAADTAVYYCAFGYSDYEYNWFDPWGQGTLVTVSSASTKGPSVFPLAPCSRSTSESTAALGCLVKDYFPEPVTVSWNSGALTSGVHTFPAVLQSSGLYSLSSVVTVPSSSLGTKTYTCNVDHKPSNTKVDKRVESKYGPPCPPCPAPEFLGGPSVFLFPPKPKDTLMISRTPEVTCVVVDVSQEDPEVQFNWYVDGVEVHNAKTKPREEQFNSTYRVVSVLTVLHQDWLNGKEYKCKVSNKGLPSSIEKTISKAKGQPREPQVYTLPPSQEEMTKNQVSLTCLVKGFYPSDIAVEWESNGQPENNYKTTPPVLDSDGSFFLYSRLTVDKSRWQEGNVFSCSVMHEALHNHYTQKSLSLSLGK

SEQ ID NO: 2 - protein, 214 aa, Artificial Sequence
  Light Chain Amino Acid Sequence; Anti-LAG-3 mAb (BMS-986016)
EIVLTQSPATLSLSPGERATLSCRASQSISSYLAWYQQKPGQAPRLLIYDASNRATGIPARFSGSGSGTDFTLTISSLEPEDFAVYYCQQRSNWPLTFGQGTNLEIKRTVAAPSVFIFPPSDEQLKSGTASVVCLLNNFYPREAKVQWKVDNALQSGNSQESVTEQDSKDSTYSLSSTLTLSKADYEKHKVYACEVTHQGLSSPVTKSFNRGEC

SEQ ID NO: 3 - protein, 120 aa, Artificial Sequence
  Heavy Chain Variable Region (VH) Amino Acid Sequence; Anti-LAG-3 mAb (BMS-986016)
QVQLQQWGAGLLKPSETLSLTCAVYGGSFSDYYWNWIRQPPGKGLEWIGEINHRGSTNSNPSLKSRVTLSLDTSKNQFSLKLRSVTAADTAVYYCAFGYSDYEYNWFDPWGQGTLVTVSS

SEQ ID NO: 4 - DNA, 360 bp, Artificial Sequence
  Heavy Chain Variable Region (VH) Nucleotide Sequence; Anti-LAG-3 mAb (BMS-986016)
caggtgcagctacagcagtggggcgcaggactgttgaagccttcggagaccctgtccctcacctgcgctgtctatggtgggtccttcagtgattactactggaactggatccgccagcccccagggaaggggctggagtggattggggaaatcaatcatcgtggaagcaccaactccaacccgtccctcaagagtcgagtcaccctatcactagacacgtccaagaaccagttctccctgaagctgaggtctgtgaccgccgcggacacggctgtgtattactgtgcgtttggatatagtgactacgagtacaactggttcgacccctggggccagggaaccctggtcaccgtctcctca

SEQ ID NO: 5 - protein, 107 aa, Artificial Sequence
  Light Chain Variable Region (VL) Amino Acid Sequence; Anti-LAG-3 mAb (BMS-986016)
EIVLTQSPATLSLSPGERATLSCRASQSISSYLAWYQQKPGQAPRLLIYDASNRATGIPARFSGSGSGTDFTLTISSLEPEDFAVYYCQQRSNWPLTFGQGTNLEIK

SEQ ID NO: 6 - DNA, 321 bp, Artificial Sequence
  Light Chain Variable Region (VL) Nucleotide Sequence; Anti-LAG-3 mAb (BMS-986016)
gaaattgtgttgacacagtctccagccaccctgtctttgtctccaggggaaagagccaccctctcctgcagggccagtcagagtattagcagctacttagcctggtaccaacagaaacctggccaggctcccaggctcctcatctatgatgcatccaacagggccactggcatcccagccaggttcagtggcagtgggtctgggacagacttcactctcaccatcagcagcctagagcctgaagattttgcagtttattactgtcagcagcgtagcaactggcctctcacttttggccaggggaccaacctggagatcaaa

SEQ ID NO: 7 - protein, 5 aa, Artificial Sequence
  Heavy Chain CDR1 Amino Acid Sequence; Anti-LAG-3 mAb (BMS-986016)
DYYWN

SEQ ID NO: 8 - protein, 16 aa, Artificial Sequence
  Heavy Chain CDR2 Amino Acid Sequence; Anti-LAG-3 mAb (BMS-986016)
EINHRGSTNSNPSLKS

SEQ ID NO: 9 - protein, 12 aa, Artificial Sequence
  Heavy Chain CDR3 Amino Acid Sequence; Anti-LAG-3 mAb (BMS-986016)
GYSDYEYNWFDP

SEQ ID NO: 10 - protein, 11 aa, Artificial Sequence
  Light Chain CDR1 Amino Acid Sequence; Anti-LAG-3 mAb (BMS-986016)
RASQSISSYLA

SEQ ID NO: 11 - protein, 7 aa, Artificial Sequence
  Light Chain CDR2 Amino Acid Sequence; Anti-LAG-3 mAb (BMS-986016)
DASNRAT

SEQ ID NO: 12 - protein, 9 aa, Artificial Sequence
  Light Chain CDR3 Amino Acid Sequence; Anti-LAG-3 mAb (BMS-986016)
QQRSNWPLT

SEQ ID NO: 13 - protein, 440 aa, Artificial Sequence
  Heavy Chain Amino Acid Sequence; Anti-PD-1 mAb (BMS936558)
QVQLVESGGGVVQPGRSLRLDCKASGITFSNSGMHWVRQAPGKGLEWVAVIWYDGSKRYYADSVKGRFTISRDNSKNTLFLQMNSLRAEDTAVYYCATNDDYWGQGTLVTVSSASTKGPSVFPLAPCSRSTSESTAALGCLVKDYFPEPVTVSWNSGALTSGVHTFPAVLQSSGLYSLSSVVTVPSSSLGTKTYTCNVDHKPSNTKVDKRVESKYGPPCPPCPAPEFLGGPSVFLFPPKPKDTLMISRTPEVTCVVVDVSQEDPEVQFNWYVDGVEVHNAKTKPREEQFNSTYRVVSVLTVLHQDWLNGKEYKCKVSNKGLPSSIEKTISKAKGQPREPQVYTLPPSQEEMTKNQVSLTCLVKGFYPSDIAVEWESNGQPENNYKTTPPVLDSDGSFFLYSRLTVDKSRWQEGNVFSCSVMHEALHNHYTQKSLSLSLGK

SEQ ID NO: 14 - protein, 213 aa, Artificial Sequence
  Light Chain Amino Acid Sequence; Anti-PD-1 mAb (BMS936558)
EIVLTQSPATLSLSPGERATLSCRASQSVSSYLAWYQQKPGQAPRLLIYDASNRATGIPARFSGSGSGTDFTLTISSLEPEDFAVYYCQQSSNWPRTFGQGTKVEIKRTVAAPSVFIFPPSDEQLKSGTASVVCLLNNFYPREAKVQWKVDNALQSGNSQESVTEQDSKDSTYSLSSTLLSKADYEKHKVYACEVTHQGLSSPVTKSFNRGEC

SEQ ID NO: 15 - protein, 113 aa, Artificial Sequence [sequence omitted]

SEQ ID NO: 16 - DNA, 339 bp, Artificial Sequence
  Heavy Chain Variable Region (VH) Nucleotide Sequence; Anti-PD-1 mAb (BMS936558)
caggtgcagctggtggagtctgggggaggcgtggtccagcctgggaggtccctgagactcgactgtaaagcgtctggaatcaccttcagtaactctggcatgcactgggtccgccaggctccaggcaaggggctggagtgggtggcagttatttggtatgatggaagtaaaagatactatgcagactccgtgaagggccgattcaccatctccagagacaattccaagaacacgctgtttctgcaaatgaacagcctgagagccgaggacacggctgtgtattactgtgcgacaaacgacgactactggggccagggaaccctggtcaccgtctcctca

SEQ ID NO: 17 - protein, 107 aa, Artificial Sequence [sequence omitted]

SEQ ID NO: 18 - DNA, 321 bp, Artificial Sequence
  Light Chain Variable Region (VL) Nucleotide Sequence; Anti-PD-1 mAb (BMS936558)
gaaattgtgttgacacagtctccagccaccctgtctttgtctccaggggaaagagccaccctctcctgcagggccagtcagagtgttagtagttacttagcctggtaccaacagaaacctggccaggctcccaggctcctcatctatgatgcatccaacagggccactggcatcccagccaggttcagtggcagtgggtctgggacagacttcactctcaccatcagcagcctagagcctgaagattttgcagtttattactgtcagcagagtagcaactggcctcggacgttcggccaagggaccaaggtggaaatcaaa

SEQ ID NO: 19 - protein, 5 aa, Artificial Sequence
  Heavy Chain CDR1 Amino Acid Sequence; Anti-PD-1 mAb (BMS936558)
NSGMH

SEQ ID NO: 20 - protein, 17 aa, Artificial Sequence
  Heavy Chain CDR2 Amino Acid Sequence; Anti-PD-1 mAb (BMS936558)
VIWYDGSKRYYADSVKG

SEQ ID NO: 21 - protein, 4 aa, Artificial Sequence
  Heavy Chain CDR3 Amino Acid Sequence; Anti-PD-1 mAb (BMS936558)
NDDY

SEQ ID NO: 22 - protein, 11 aa, Artificial Sequence
  Light Chain CDR1 Amino Acid Sequence; Anti-PD-1 mAb (BMS936558)
RASQSVSSYLA

SEQ ID NO: 23 - protein, 7 aa, Artificial Sequence
  Light Chain CDR2 Amino Acid Sequence; Anti-PD-1 mAb (BMS936558)
DASNRAT

SEQ ID NO: 24 - protein, 9 aa, Artificial Sequence
  Light Chain CDR3 Amino Acid Sequence; Anti-PD-1 mAb (BMS936558)
QQSSNWPRT

SEQ ID NO: 25 - DNA, 1344 bp, Artificial Sequence
  Heavy Chain Nucleotide Sequence; Anti-LAG-3 mAb (BMS-986016)
caggtgcagctacagcagtggggcgcaggactgttgaagccttcggagaccctgtccctcacctgcgctgtctatggtgggtccttcagtgattactactggaactggatccgccagcccccagggaaggggctggagtggattggggaaatcaatcatcgtggaagcaccaactccaacccgtccctcaagagtcgagtcaccctatcactagacacgtccaagaaccagttctccctgaagctgaggtctgtgaccgccgcggacacggctgtgtattactgtgcgtttggatatagtgactacgagtacaactggttcgacccctggggccagggaaccctggtcaccgtctcctcagctagcaccaagggcccatccgtcttccccctggcgccctgctccaggagcacctccgagagcacagccgccctgggctgcctggtcaaggactacttccccgaaccggtgacggtgtcgtggaactcaggcgccctgaccagcggcgtgcacaccttcccggctgtcctacagtcctcaggactctactccctcagcagcgtggtgaccgtgccctccagcagcttgggcacgaagacctacacctgcaacgtagatcacaagcccagcaacaccaaggtggacaagagagttgagtccaaatatggtcccccatgcccaccatgcccagcacctgagttcctggggggaccatcagtcttcctgttccccccaaaacccaaggacactctcatgatctcccggacccctgaggtcacgtgcgtggtggtggacgtgagccaggaagaccccgaggtccagttcaactggtacgtggatggcgtggaggtgcataatgccaagacaaagccgcgggaggagcagttcaacagcacgtaccgtgtggtcagcgtcctcaccgtcctgcaccaggactggctgaacggcaaggagtacaagtgcaaggtctccaacaaaggcctcccgtcctccatcgagaaaaccatctccaaagccaaagggcagccccgagagccacaggtgtacaccctgcccccatcccaggaggagatgaccaagaaccaggtcagcctgacctgcctggtcaaaggcttctaccccagcgacatcgccgtggagtgggagagcaatgggcagccggagaacaactacaagaccacgcctcccgtgctggactccgacggctccttcttcctctacagcaggctaaccgtggacaagagcaggtggcaggaggggaatgtcttctcatgctccgtgatgcatgaggctctgcacaaccactacacacagaagagcctctccctgtctctgggtaaatga

SEQ ID NO: 26 - DNA, 645 bp, Artificial Sequence
  Light Chain Nucleotide Sequence; Anti-LAG-3 mAb (BMS-986016)
gaaattgtgttgacacagtctccagccaccctgtctttgtctccaggggaaagagccaccctctcctgcagggccagtcagagtattagcagctacttagcctggtaccaacagaaacctggccaggctcccaggctcctcatctatgatgcatccaacagggccactggcatcccagccaggttcagtggcagtgggtctgggacagacttcactctcaccatcagcagcctagagcctgaagattttgcagtttattactgtcagcagcgtagcaactggcctctcacttttggccaggggaccaacctggagatcaaacgtacggtggctgcaccatctgtcttcatcttcccgccatctgatgagcagttgaaatctggaactgcctctgttgtgtgcctgctgaataacttctatcccagagaggccaaagtacagtggaaggtggataacgccctccaatcgggtaactcccaggagagtgtcacagagcaggacagcaaggacagcacctacagcctcagcagcaccctgacgctgagcaaagcagactacgagaaacacaaagtctacgcctgcgaagtcacccatcagggcctgagctcgcccgtcacaaagagcttcaacaggggagagtgttag

SEQ ID NO: 27 - protein, 8 aa, Artificial Sequence
  human LAG-3 binding epitope
PGHPLAPG

SEQ ID NO: 28 - protein, 8 aa, Artificial Sequence
  human LAG-3 binding epitope
HPAAPSSW

SEQ ID NO: 29 - protein, 8 aa, Artificial Sequence
  human LAG-3 binding epitope
PAAPSSWG

SEQ ID NO: 30 - protein, 446 aa, Artificial Sequence
  Heavy Chain Amino Acid Sequence; Anti-LAG-3 mAb (BMS-986016)
QVQLQQWGAGLLKPSETLSLTCAVYGGSFSDYYWNWIRQPPGKGLEWIGEINHRGSTNSNPSLKSRVTLSLDTSKNQFSLKLRSVTAADTAVYYCAFGYSDYEYNWFDPWGQGTLVTVSSASTKGPSVFPLAPCSRSTSESTAALGCLVKDYFPEPVTVSWNSGALTSGVHTFPAVLQSSGLYSLSSVVTVPSSSLGTKTYTCNVDHKPSNTKVDKRVESKYGPPCPPCPAPEFLGGPSVFLFPPKPKDTLMISRTPEVTCVVVDVSQEDPEVQFNWYVDGVEVHNAKTKPREEQFNSTYRVVSVLTVLHQDWLNGKEYKCKVSNKGLPSSIEKTISKAKGQPREPQVYTLPPSQEEMTKNQVSLTCLVKGFYPSDIAVEWESNGQPENNYKTTPPVLDSDGSFFLYSRLTVDKSRWQEGNVFSCSVMHEALHNHYTQKSLSLSLG